European Patent Application EP 4 265 632 A1, published October 25, 2023. Title: SELF-ASSEMBLED NANOPARTICLE CONTAINING gHgL PROTEIN OF EB VIRUS, PREPARATION METHOD AND USE THEREOF. Applicant: SUN YAT-SEN UNIVERSITY Sun Yat-sen University Cancer Center(SYSUCC). The sequence listing filed with the application follows.

SEQUENCE LISTING (38 sequences)

SEQ ID NO: 1 - protein, 789 aa, Artificial Sequence
  synthesized
WAYPCCHVTQLRAQHLLALENISDIYLVSNQTCDGFSLASLNSPKNGSNQLVISRCANGLNVVSFFISILKRSSSALTSHLRELLTTLESLYGSFSVEDLFGANLNRYAWHRGGGGGGSGGGGSGGGGSSLSEVKLHLDIEGHASHYTIPWTELMAKVPGLSPEALWREANVTEDLASMLNRYKLIYKTSGTLGIALAEPVDIPAVSEGSMQVDASKVHPGVISGLNSPACMLSAPLEKQLFYYIGTMLPNTRPHSYVFYQLRCHLSYVALSINGDKFQYTGAMTSKFLMGTYKRVTEKGDEHVLSLIFGKTKDLPDLRGPFSYPSLTSAQSGDYSLVIVTTFVHYANFHNYFVPNLKDMFSRAVTMTAASYARYVLQKLVLLEMKGGCREPELDTETLTTMFEVSVAFFKVGHAVGETGNGCVDLRWLAKSFFELTVLKDIIGICYGATVKGMQSYGLERLAAMLMATVKMEELGHLTTEKQEYALRLATVGYPKAGVYSGLIGGATSVLLSAYNRHPLFQPLHTVMRETLFIGSHVVLRELRLNVTTQGPNLALYQLLSTALCSALEIGEVLRGLALGTESGLFSPCYLSLRFDLTRDKLLSMAPQEAMLDQAAVSNAVDGFLGRLSLEREDRDAWHLPAYKCVDRLDKVLMIIPLINVTFIISSDREVRGSALYEASTTYLSSSLFLSPVIMNKCSQGAVAGEPRQIPKIQNFTRTQKSCIFCGFALLSYDEKEGLETTTYITSQEVQNSILSSNYFDFDNLHVHYLLLTTNGTVMEIAGLYEERA

SEQ ID NO: 2 - DNA, 342 bp, Epstein-Barr Virus
tgggcatatccatgctgtcacgtgacccagctgagggcacagcacctgctggccctggagaatatctctgacatctacctggtgagcaaccagacatgcgatggcttctctctggccagcctgaacagccccaagaacggctccaatcagctggtcatctctcgctgtgccaacggcctgaatgtggtgtctttctttatcagcatcctgaagcggagctcctctgccctgacctcccacctgagagagctgctgaccacactggagtctctgtacggcagcttttccgtggaggacctgttcggcgccaacctgaatcggtatgcctggcacagaggagga

SEQ ID NO: 3 - DNA, 45 bp, Artificial Sequence
  synthesized
ggaggaggaggatctggaggaggaggcagcggcggcggcggcagc

SEQ ID NO: 4 - DNA, 1980 bp, Epstein-Barr Virus
tccctgagcgaggtgaagctgcacctggacatcgagggccacgcctcccactacacaatcccctggaccgagctgatggccaaggtgccaggactgtccccagaggccctgtggcgggaggccaatgtgaccgaggatctggcctctatgctgaacagatacaagctgatctataagacaagcggcaccctgggaatcgccctggcagagcctgtggacatcccagccgtgtctgagggcagcatgcaggtggatgcctccaaggtgcaccctggcgtgatctccggcctgaactctcctgcctgcatgctgtctgccccactggagaagcagctgttttactatatcggcacaatgctgcccaataccaggcctcacagctacgtgttctatcagctgcgctgtcacctgtcctacgtggccctgtctatcaacggcgacaagtttcagtatacaggcgccatgaccagcaagttcctgatgggcacatacaagcgggtgaccgagaagggcgatgagcacgtgctgtccctgatctttggcaagacaaaggacctgcccgatctgagaggcccattctcctacccctctctgaccagcgcccagtccggcgactattccctggtcatcgtgaccacatttgtgcactacgccaactttcacaattatttcgtgcccaatctgaaggatatgttcagcagggccgtgacaatgaccgcagcatcctacgcaagatatgtgctgcagaagctggtgctgctggagatgaagggcggctgtcgggagcctgagctggatacagagaccctgaccacaatgtttgaggtgagcgtggccttctttaaagtgggacacgcagtgggagagacaggaaacggctgcgtggacctgagatggctggccaagtctttctttgagctgacagtgctgaaggatatcatcggcatctgttacggcgccaccgtgaagggcatgcagagctatggcctggagaggctggccgccatgctgatggccaccgtgaagatggaggagctgggccacctgaccacagagaagcaggagtacgcactgaggctggcaacagtgggataccctaaggcaggcgtgtattccggactgatcggaggagccaccagcgtgctgctgtccgcctataatcggcaccctctgtttcagccactgcacacagtgatgagagagaccctgttcatcggaagccacgtggtgctgagggagctgcgcctgaatgtgaccacacagggcccaaacctggccctgtaccagctgctgagcaccgccctgtgctccgccctggagatcggagaggtgctgaggggactggccctgggcacagagtctggcctgtttagcccatgttatctgtccctgaggttcgacctgactcgcgataagctgctgtctatggcaccacaggaggcaatgctggaccaggcagccgtgagcaatgccgtggatggcttcctgggcaggctgtccctggagagggaggacagagatgcctggcacctgcccgcctacaagtgcgtggaccgcctggataaggtgctgatgatcatccctctgatcaacgtgacctttatcatctctagcgacagggaggtgcgcggaagcgccctgtacgaggcctccaccacatatctgtcctctagcctgttcctgtcccccgtgatcatgaataagtgttctcagggagcagtggcaggagagccaaggcagatccctaagatccagaactttacaagaacccagaagtcttgcatcttttgtggcttcgccctgctgagctacgatgagaaggagggcctggagaccacaacctatatcacatctcaggaggtgcagaacagcatcctgtcctctaattacttcgactttgataacctgcacgtgcactatctgctgctgacaaccaacggcaccgtgatggagatcgccggcctgtacgaggagagggca

SEQ ID NO: 5 - DNA, 81 bp, Artificial Sequence
  synthesized
ggatacatcccagaggcaccaagggacggacaggcctatgtgcgcaaggatggcgagtgggtgctgctgtctaccttcctg

SEQ ID NO: 6 - DNA, 627 bp, Artificial Sequence
  synthesized
atgaagatggaggagctgtttaagaagcacaagatcgtggccgtgctgagggccaactccgtggaggaggccatcgagaaggcagtggccgtgttcgcaggaggagtgcacctgatcgagatcacctttacagtgcctgacgccgatacagtgatcaaggccctgagcgtgctgaaggagaagggagcaatcatcggagcaggaaccgtgacatccgtggagcagtgcaggaaggcagtggagtccggagccgagttcatcgtgtctccccacctggacgaggagatctctcagttctgtaaggagaagggcgtgttttacatgcctggcgtgatgaccccaacagagctggtgaaggccatgaagctgggccacgatatcctgaagctgttcccaggagaggtggtgggacctcagtttgtgaaggccatgaagggccccttccctaatgtgaagtttgtgccaaccggcggcgtgaacctggacaacgtgtgcgagtggttcaaggcaggcgtgctggcagtgggagtgggcgatgccctggtgaagggcgaccccgatgaggtgagggagaaggccaagaagtttgtggagaagatccgcggctgtacagagggctccctggag

SEQ ID NO: 7 - DNA, 15 bp, Artificial Sequence
  synthesized
ggaggaagcggaagc

SEQ ID NO: 8 - DNA, 18 bp, Artificial Sequence
  synthesized
ggaggaagcggaggctct

SEQ ID NO: 9 - DNA, 21 bp, Artificial Sequence
  synthesized
ggaggaagcggaggctctgga

SEQ ID NO: 10 - DNA, 24 bp, Artificial Sequence
  synthesized
ggaggaagcggaggctctggaagc

SEQ ID NO: 11 - DNA, 27 bp, Artificial Sequence
  synthesized
ggaggaagcggaggctctggaggctct

SEQ ID NO: 12 - protein, 5 aa, Artificial Sequence
  synthesized
GGSGS

SEQ ID NO: 13 - protein, 6 aa, Artificial Sequence
  synthesized
GGSGGS

SEQ ID NO: 14 - protein, 7 aa, Artificial Sequence
  synthesized
GGSGGSG

SEQ ID NO: 15 - protein, 8 aa, Artificial Sequence
  synthesized
GGSGGSGS

SEQ ID NO: 16 - protein, 9 aa, Artificial Sequence
  synthesized
GGSGGSGGS

SEQ ID NO: 17 - DNA, 54 bp, Artificial Sequence
  synthesized
ggaggaagcggaggctctggaagcgagaaggcagcaaaggcagaggaggcagcc

SEQ ID NO: 18 - DNA, 72 bp, Artificial Sequence
  synthesized
atgccaatgggctctctgcagcccctggccacactgtacctgctgggaatgctggtggcaagctgcctggga

SEQ ID NO: 19 - DNA, 24 bp, Artificial Sequence
  synthesized
catcatcaccaccaccaccaccac

SEQ ID NO: 20 - DNA, 12 bp, Artificial Sequence
  synthesized
ggaagcggatcc

SEQ ID NO: 21 - DNA, 3237 bp, Artificial Sequence
  synthesized
atgccaatgggctctctgcagcccctggccacactgtacctgctgggaatgctggtggcaagctgcctgggatgggcatatccatgctgtcacgtgacccagctgagggcacagcacctgctggccctggagaatatctctgacatctacctggtgagcaaccagacatgcgatggcttctctctggccagcctgaacagccccaagaacggctccaatcagctggtcatctctcgctgtgccaacggcctgaatgtggtgtctttctttatcagcatcctgaagcggagctcctctgccctgacctcccacctgagagagctgctgaccacactggagtctctgtacggcagcttttccgtggaggacctgttcggcgccaacctgaatcggtatgcctggcacagaggaggaggaggaggaggatctggaggaggaggcagcggcggcggcggcagctccctgagcgaggtgaagctgcacctggacatcgagggccacgcctcccactacacaatcccctggaccgagctgatggccaaggtgccaggactgtccccagaggccctgtggcgggaggccaatgtgaccgaggatctggcctctatgctgaacagatacaagctgatctataagacaagcggcaccctgggaatcgccctggcagagcctgtggacatcccagccgtgtctgagggcagcatgcaggtggatgcctccaaggtgcaccctggcgtgatctccggcctgaactctcctgcctgcatgctgtctgccccactggagaagcagctgttttactatatcggcacaatgctgcccaataccaggcctcacagctacgtgttctatcagctgcgctgtcacctgtcctacgtggccctgtctatcaacggcgacaagtttcagtatacaggcgccatgaccagcaagttcctgatgggcacatacaagcgggtgaccgagaagggcgatgagcacgtgctgtccctgatctttggcaagacaaaggacctgcccgatctgagaggcccattctcctacccctctctgaccagcgcccagtccggcgactattccctggtcatcgtgaccacatttgtgcactacgccaactttcacaattatttcgtgcccaatctgaaggatatgttcagcagggccgtgacaatgaccgcagcatcctacgcaagatatgtgctgcagaagctggtgctgctggagatgaagggcggctgtcgggagcctgagctggatacagagaccctgaccacaatgtttgaggtgagcgtggccttctttaaagtgggacacgcagtgggagagacaggaaacggctgcgtggacctgagatggctggccaagtctttctttgagctgacagtgctgaaggatatcatcggcatctgttacggcgccaccgtgaagggcatgcagagctatggcctggagaggctggccgccatgctgatggccaccgtgaagatggaggagctgggccacctgaccacagagaagcaggagtacgcactgaggctggcaacagtgggataccctaaggcaggcgtgtattccggactgatcggaggagccaccagcgtgctgctgtccgcctataatcggcaccctctgtttcagccactgcacacagtgatgagagagaccctgttcatcggaagccacgtggtgctgagggagctgcgcctgaatgtgaccacacagggcccaaacctggccctgtaccagctgctgagcaccgccctgtgctccgccctggagatcggagaggtgctgaggggactggccctgggcacagagtctggcctgtttagcccatgttatctgtccctgaggttcgacctgactcgcgataagctgctgtctatggcaccacaggaggcaatgctggaccaggcagccgtgagcaatgccgtggatggcttcctgggcaggctgtccctggagagggaggacagagatgcctggcacctgcccgcctacaagtgcgtggaccgcctggataaggtgctgatgatcatccctctgatcaacgtgacctttatcatctctagcgacagggaggtgcgcggaagcgccctgtacgaggcctccaccacatatctgtcctctagcctgttcctgtcccccgtgatcatgaataagtgttctcagggagcagtggcaggagagccaaggcagatccctaagatccagaactttacaagaacccagaagtcttgcatcttttgtggcttcgccctgctgagctacgatgagaaggagggcctggagaccacaacctatatcacatctcaggaggtgcagaacagcatcctgtcctctaattacttcgactttgataacctgcacgtgcactatctgctgctgacaaccaacggcaccgtgatggagatcgccggcctgtacgaggagagggcaggatacatcccagaggcaccaagggacggacaggcctatgtgcgcaaggatggcgagtgggtgctgctgtctaccttcctgggaagcggatcccatcatcaccaccaccaccaccacggaggaagcggaggctctggaagcgagaaggcagcaaaggcagaggaggcagccatgaagatggaggagctgtttaagaagcacaagatcgtggccgtgctgagggccaactccgtggaggaggccatcgagaaggcagtggccgtgttcgcaggaggagtgcacctgatcgagatcacctttacagtgcctgacgccgatacagtgatcaaggccctgagcgtgctgaaggagaagggagcaatcatcggagcaggaaccgtgacatccgtggagcagtgcaggaaggcagtggagtccggagccgagttcatcgtgtctccccacctggacgaggagatctctcagttctgtaaggagaagggcgtgttttacatgcctggcgtgatgaccccaacagagctggtgaaggccatgaagctgggccacgatatcctgaagctgttcccaggagaggtggtgggacctcagtttgtgaaggccatgaagggccccttccctaatgtgaagtttgtgccaaccggcggcgtgaacctggacaacgtgtgcgagtggttcaaggcaggcgtgctggcagtgggagtgggcgatgccctggtgaagggcgaccccgatgaggtgagggagaaggccaagaagtttgtggagaagatccgcggctgtacagagggctccctggag

SEQ ID NO: 22 - DNA, 483 bp, Artificial Sequence
  synthesized
atgaaccagcacagccacaaggaccacgagaccgtgcgtattgcggtggttcgtgcgcgttggcatgcggagattgtggatgcgtgcgttagcgcgttcgaagcggcgatgcgtgacatcggtggcgatcgtttcgcggtggacgtttttgatgtgccgggtgcgtacgagattccgctgcatgcgcgtaccctggcggaaaccggtcgttatggcgcggttctgggcaccgcgttcgtggttaacggtggcatctaccgtcacgaatttgtggcgagcgcggttattaacggtatgatgaacgtgcaactgaacaccggcgtgccggttctgagcgcggttctgaccccgcacaactatgacaagagcaaagcgcacaccctgctgttcctggcgctgtttgcggtgaagggtatggaagcggcgcgtgcgtgcgttgagatcctggcggcgcgtgaaaaaattgcggcgggcagcctggaa

SEQ ID NO: 23 - DNA, 18 bp, Artificial Sequence
  synthesized
catcatcaccaccaccac

SEQ ID NO: 24 - protein, 167 aa, Artificial Sequence
  synthesized
MNQHSHKDHETVRIAVVRARWHAEIVDACVSAFEAAMRDIGGDRFAVDVFDVPGAYEIPLHARTLAETGRYGAVLGTAFVVNGGIYRHEFVASAVINGMMNVQLNTGVPVLSAVLTPHNYDKSKAHTLLFLALFAVKGMEAARACVEILAAREKIAAGSLEHHHHHH

SEQ ID NO: 25 - protein, 1055 aa, Artificial Sequence
  synthesized
WAYPCCHVTQLRAQHLLALENISDIYLVSNQTCDGFSLASLNSPKNGSNQLVISRCANGLNVVSFFISILKRSSSALTSHLRELLTTLESLYGSFSVEDLFGANLNRYAWHRGGGGGGSGGGGSGGGGSSLSEVKLHLDIEGHASHYTIPWTELMAKVPGLSPEALWREANVTEDLASMLNRYKLIYKTSGTLGIALAEPVDIPAVSEGSMQVDASKVHPGVISGLNSPACMLSAPLEKQLFYYIGTMLPNTRPHSYVFYQLRCHLSYVALSINGDKFQYTGAMTSKFLMGTYKRVTEKGDEHVLSLIFGKTKDLPDLRGPFSYPSLTSAQSGDYSLVIVTTFVHYANFHNYFVPNLKDMFSRAVTMTAASYARYVLQKLVLLEMKGGCREPELDTETLTTMFEVSVAFFKVGHAVGETGNGCVDLRWLAKSFFELTVLKDIIGICYGATVKGMQSYGLERLAAMLMATVKMEELGHLTTEKQEYALRLATVGYPKAGVYSGLIGGATSVLLSAYNRHPLFQPLHTVMRETLFIGSHVVLRELRLNVTTQGPNLALYQLLSTALCSALEIGEVLRGLALGTESGLFSPCYLSLRFDLTRDKLLSMAPQEAMLDQAAVSNAVDGFLGRLSLEREDRDAWHLPAYKCVDRLDKVLMIIPLINVTFIISSDREVRGSALYEASTTYLSSSLFLSPVIMNKCSQGAVAGEPRQIPKIQNFTRTQKSCIFCGFALLSYDEKEGLETTTYITSQEVQNSILSSNYFDFDNLHVHYLLLTTNGTVMEIAGLYEERAGYIPEAPRDGQAYVRKDGEWVLLSTFLGSGSHHHHHHHHGGSGGSGSEKAAKAEEAAMKMEELFKKHKIVAVLRANSVEEAIEKAVAVFAGGVHLIEITFTVPDADTVIKALSVLKEKGAIIGAGTVTSVEQCRKAVESGAEFIVSPHLDEEISQFCKEKGVFYMPGVMTPTELVKAMKLGHDILKLFPGEVVGPQFVKAMKGPFPNVKFVPTGGVNLDNVCEWFKAGVLAVGVGDALVKGDPDEVREKAKKFVEKIRGCTEGSLE

SEQ ID NO: 26 - protein, 209 aa, Artificial Sequence
  synthesized
MKMEELFKKHKIVAVLRANSVEEAIEKAVAVFAGGVHLIEITFTVPDADTVIKALSVLKEKGAIIGAGTVTSVEQCRKAVESGAEFIVSPHLDEEISQFCKEKGVFYMPGVMTPTELVKAMKLGHDILKLFPGEVVGPQFVKAMKGPFPNVKFVPTGGVNLDNVCEWFKAGVLAVGVGDALVKGDPDEVREKAKKFVEKIRGCTEGSLE

SEQ ID NO: 27 - protein, 161 aa, Artificial Sequence
  synthesized
MNQHSHKDHETVRIAVVRARWHAEIVDACVSAFEAAMRDIGGDRFAVDVFDVPGAYEIPLHARTLAETGRYGAVLGTAFVVNGGIYRHEFVASAVINGMMNVQLNTGVPVLSAVLTPHNYDKSKAHTLLFLALFAVKGMEAARACVEILAAREKIAAGSLE

SEQ ID NO: 28 - protein, 114 aa, Epstein-Barr Virus
WAYPCCHVTQLRAQHLLALENISDIYLVSNQTCDGFSLASLNSPKNGSNQLVISRCANGLNVVSFFISILKRSSSALTSHLRELLTTLESLYGSFSVEDLFGANLNRYAWHRGG

SEQ ID NO: 29 - protein, 660 aa, Epstein-Barr Virus
SLSEVKLHLDIEGHASHYTIPWTELMAKVPGLSPEALWREANVTEDLASMLNRYKLIYKTSGTLGIALAEPVDIPAVSEGSMQVDASKVHPGVISGLNSPACMLSAPLEKQLFYYIGTMLPNTRPHSYVFYQLRCHLSYVALSINGDKFQYTGAMTSKFLMGTYKRVTEKGDEHVLSLIFGKTKDLPDLRGPFSYPSLTSAQSGDYSLVIVTTFVHYANFHNYFVPNLKDMFSRAVTMTAASYARYVLQKLVLLEMKGGCREPELDTETLTTMFEVSVAFFKVGHAVGETGNGCVDLRWLAKSFFELTVLKDIIGICYGATVKGMQSYGLERLAAMLMATVKMEELGHLTTEKQEYALRLATVGYPKAGVYSGLIGGATSVLLSAYNRHPLFQPLHTVMRETLFIGSHVVLRELRLNVTTQGPNLALYQLLSTALCSALEIGEVLRGLALGTESGLFSPCYLSLRFDLTRDKLLSMAPQEAMLDQAAVSNAVDGFLGRLSLEREDRDAWHLPAYKCVDRLDKVLMIIPLINVTFIISSDREVRGSALYEASTTYLSSSLFLSPVIMNKCSQGAVAGEPRQIPKIQNFTRTQKSCIFCGFALLSYDEKEGLETTTYITSQEVQNSILSSNYFDFDNLHVHYLLLTTNGTVMEIAGLYEERA

SEQ ID NO: 30 - protein, 15 aa, Artificial Sequence
  synthesized
GGGGSGGGGSGGGGS

SEQ ID NO: 31 - protein, 10 aa, Artificial Sequence
  synthesized
EKAAKAEEAA

SEQ ID NO: 32 - protein, 27 aa, Artificial Sequence
  synthesized
GYIPEAPRDGQAYVRKDGEWVLLSTFL

SEQ ID NO: 33 - protein, 32 aa, Artificial Sequence
  synthesized
MKQIEDKIEEILSKIYHIENEIARIKKLIGEV

SEQ ID NO: 34 - protein, 8 aa, Artificial Sequence
  synthesized
HHHHHHHH

SEQ ID NO: 35 - protein, 6 aa, Artificial Sequence
  synthesized
HHHHHH

SEQ ID NO: 36 - protein, 24 aa, Artificial Sequence
  synthesized
MPMGSLQPLATLYLLGMLVASCLG

SEQ ID NO: 37 - protein, 4 aa, Artificial Sequence
  synthesized
GSGS

SEQ ID NO: 38 - protein, 797 aa, Artificial Sequence
  synthesized
WAYPCCHVTQLRAQHLLALENISDIYLVSNQTCDGFSLASLNSPKNGSNQLVISRCANGLNVVSFFISILKRSSSALTSHLRELLTTLESLYGSFSVEDLFGANLNRYAWHRGGGGGGSGGGGSGGGGSSLSEVKLHLDIEGHASHYTIPWTELMAKVPGLSPEALWREANVTEDLASMLNRYKLIYKTSGTLGIALAEPVDIPAVSEGSMQVDASKVHPGVISGLNSPACMLSAPLEKQLFYYIGTMLPNTRPHSYVFYQLRCHLSYVALSINGDKFQYTGAMTSKFLMGTYKRVTEKGDEHVLSLIFGKTKDLPDLRGPFSYPSLTSAQSGDYSLVIVTTFVHYANFHNYFVPNLKDMFSRAVTMTAASYARYVLQKLVLLEMKGGCREPELDTETLTTMFEVSVAFFKVGHAVGETGNGCVDLRWLAKSFFELTVLKDIIGICYGATVKGMQSYGLERLAAMLMATVKMEELGHLTTEKQEYALRLATVGYPKAGVYSGLIGGATSVLLSAYNRHPLFQPLHTVMRETLFIGSHVVLRELRLNVTTQGPNLALYQLLSTALCSALEIGEVLRGLALGTESGLFSPCYLSLRFDLTRDKLLSMAPQEAMLDQAAVSNAVDGFLGRLSLEREDRDAWHLPAYKCVDRLDKVLMIIPLINVTFIISSDREVRGSALYEASTTYLSSSLFLSPVIMNKCSQGAVAGEPRQIPKIQNFTRTQKSCIFCGFALLSYDEKEGLETTTYITSQEVQNSILSSNYFDFDNLHVHYLLLTTNGTVMEIAGLYEERAHHHHHHHH